European Patent Application EP 4 130 261 A1, published February 8, 2023. Title: Buffer composition for purification of nucleic acid with a column based one-tube PCR and use thereof. Applicant: Gene2us Co. Soonchunhyang University Industry Academy Cooperation Foundation. The sequence listing filed with the application follows.

SEQUENCE LISTING (4 sequences)

SEQ ID NO: 1 - DNA, 20 bp, Artificial Sequence
  GAPDH forward primer
tgcaccaccaactgcttagc

SEQ ID NO: 2 - DNA, 21 bp, Artificial Sequence
  GAPDH reverse primer
cgcatggactgtggtcatgag

SEQ ID NO: 3 - DNA, 20 bp, Artificial Sequence
  uidA forward primer
tatggaatttcgccgatttt

SEQ ID NO: 4 - DNA, 20 bp, Artificial Sequence
  uidA reverse primer
tgtttgcctccctgctgcgg